European Patent Specification EP 3 785 033 B1, published December 10, 2025. Title: Intestinal and fecal biomarkers for intestinal health of poultry. Applicant: Universiteit Gent. The sequence listing filed with the application follows.

SEQUENCE LISTING (255 sequences)

SEQ ID NO: 1 - protein, 326 aa, Gallus gallus
QGKGEKHKGVDVICTDGSIVYAPFSGQLSGPIRFFHNGNAIDDGVQISGSGYCVKLVCIHPIRYHGQIQKGQQLGRMLPMQKVFPGIVSHIHVENCDQSDPTHLLRPIPDISPPFPQQDAHWAVVCAGNPTNEIRGCDKYGCGYFGAPRRNGKGEKHKGVDVICADGATVYAPFSGELSGPVKFFHNGNAIDDGVQIRGSGFCVKLLCIHPIRYNGRISKGQVLGRMLPMQRVFPGIISHMPALSLIALLSLVSTAFARQWEVHPPQQQGRHWAQICSGNPFNRIRGCDRYGCGNYGASRIHVENCDRSDPTSNLERGKGESEMEV

SEQ ID NO: 2 - protein, 1256 aa, Gallus gallus
PLDQCQDSETRTFYQIGDSWEKYVHGVRYQCYCYGRGIGEWHCQPLQAYAPLSPPTNLRLEPNPDTGILIVSWDRSTTPGISGYRVTTAPTNGQQGSTLEEVVGADQTSCTFENLNPGVEYNVSVYAVKDDQESIPISKTITQEVPQLTDLSFVDITDSSIGLRWTPLNASTIIGYRITVVAAGESVPIFEDFVDSSVGYYTVTGLEPGIDYDISVITLINGGESAPTTLTQQTAVPPPTDLRFTNVGPDTMRVTWTAPTSIVLSSFLVRYSPVKKEEDVAELTISPSDNVVVLTNLLPGTEYLVRVYSVAEQHESAPLSGIQKTGLDSPTGLDFSDITANSFTVHWIAPRATITGYKIRHHPEHGVGRPKEDRVPPSRNSITLTNLLPGTEYVVSIIAVNGREESVPLVGQQTTVSDVPRDLEVNPTSPTSLEISWDAPAVTVRYYRITYGETGGSSPVQEFTVPGTMSRATITGLKPGVDYTITVYAVTGRGDSPASSKPVTVTYKTEIDTPSQMQVTDVQDNSISIRWLPSSSPVTGYRVTAVPKKGHGPTKTKNVPPDQTQVTIEGLQPTVEYMVSVYAQNQNGESLPLVETAVTNIDRPKGLTFTEVDVDSIKIAWESPQGQVTRYRVTYSSPEDGIHELLPAPGGEEDTAELHGLRPGSEYTINIVAIYDDMESLPLTGTQSTAIPPPTNLKFTQVTPTSLTVNWNAPNVRLTGYRVRVNPKEKTGPMKEINLSPDSTSAVVSGLMVATKYEVSVYALKDSLTSRPAQGVVTTLENVSPPRRARVTDATETTITITWRTKTETITGFQIDAIPAASGQNPIQRTISPDVRTYTITGLQPGNDYKIYLYTLNENARSSPVVIDASTAIDAPSNLRFLTTTTNSLLASWQPPRAKITGYIIRYDKPGSPAKELLPRPRPGTTEATITGLEPGTEYTIYIIAVKNNQKSEPLVGRKRTDDLPTLITGPHPNQPDMLDVPSVDEGTPYLTNNRYDNGNGIQLPGTSGHPQTIGHQGQQVFFEEHGYRRPVPTTATPLRPGSRRQPPNVDEAIEIPGYQVPIIVVPSYPHSREPRRNDTTGQEALSQTTISWRPLLESTEYIISCQPVSQDEDTLQFRVPGTSSSATLTGLTRGATYNIIVEALKDHRRQKVLEEVVTVGNTVSEGLNQPADDTCYDTYTGSFYSIGEEWERLSETGFKLWCQCLGFGSGHFRCDSSKWCHDNGVNYKIGEKWDRQGENGQMIDCTCLGNGKGEF

SEQ ID NO: 3 - protein, 321 aa, Gallus gallus
MAKYTRGTVTAFSPFDARADAEALRKAMKGMGTDEETILKILTSRNNAQRQEIASAFKTLFGRDLVDDLKSELTGKFETLMVSLMRPARIFDAHALKHAIKGAGTNEKVLTEILASRTPAEVQNIKQVYMQEYEANLEDKITGETSGHFQRLLVVLLQANRDPDGRVDEALVEKDAQVLFRAGELKWGTDEETFITILGTRSVSHLRRVFDKYMTISGFQIEETIDRETSGDLEKLLLAVVKCIRSVPAYFAETLYYSMKGAGTDDDTLIRVMVSRSEIDLLDIRHEFRKNFAKSLYQMIQKDTSGDYRKALLLLCGGDDE

SEQ ID NO: 4 - protein, 294 aa, Gallus gallus
MEDSAMDMESMGPLRPQTFLFGCELKAEKEYQFKVDDEENEHQLSLRTVTLGAGAKDELHVVEAEALDYEGNPTKVVLASLKMSVQPTVSLGGFEITPPFVLRLKCGSGPVYVSGQHLVALEEEPESEDEEEDTKIGNASTKRPASGGGAKTPQKKPKLSEDDEDDDEDEDDDEDDEDDLDDDEEEIKTPMKKPAREPAGKNMQKAKQNGKDSKPSTPASKTKTPDSKKDKSLTPKTPKVPLSLEEIKAKMQASVDKGCSLPKLEPKFANYVKNCFRTEDQKVIQALWQWRQTL

SEQ ID NO: 5 - protein, 260 aa, Gallus gallus
MSHHWGYDSHNGPAHWHEHFPIANGERQSPIAISTKAARYDPALKPLSFSYDAGTAKAIVNNGHSFNVEFDDSSDKSVLQGGALDGVYRLVQFHIHWGSCEGQGSEHTVDGVKYDAELHIVHWNVKYGKFAEALKHPDGLAVVGIFMKVGNAKPEIQKVVDALNSIQTKGKQASFTNFDPTGLLPPCRDYWTYPGSLTTPPLHECVIWHVLKEPITVSSEQMCKLRGLCFSAENEPVCRMVDNWRPCQPLKSREVRASFQ

SEQ ID NO: 6 - protein, 972 aa, Gallus gallus
MAAGFFISKSVGIVGIVLALGAVATIIALSVVYAQEKNKSSGGSGGSDTTSTTTASTTTTSTTTASTTAAPNNPWNRWRLPTALKPESYEVTLQPFLTPDDNNMYIFKGNSSVVFLCEEATDLILIHSNKLNYTLQGGFHASLHAVNGSTPPTISNTWLETNTQYLVLQLAGPLQQGQHYRLFSIFTGELADDLAGFYRSEYTEGNVTKVVATTQMQAPDARKAFPCFDEPAMKAVFTVTMIHPSDHTAISNMPVHSTYQLQMDGQSWNVTQFDPTPRMSTYLLAFIVSQFDYVENNTGKVQIRIWGRPAAIAEGQGEYALEKTGPILSFFERHYNTAYPLPKSDQVGLPDFNAGAMENWGLVTYRENSLLYDNAYSSIGNKERVVTVIAHELAHQWFGNLVTLRWWNDLWLNEGFASYVEYLGADSAEPTWDIKDLMVLNELYTVMATDALTTSHPLTFREDEINTPAQISEVFDSIAYSKGASVLRMLSDFLTEDVFKEGLQSYLHDFSYNNTVYTDLWDHLQEAVNKNSVPLPDSIGAIMDRWTLQMGFPVVTVNTLTGSVQQSHFLLDSNSTVERPSVFNYTWIVPITWMTPSRTGDRYWLVDVSATNSDFSVGSSTWLLLNLNVSGYFRVNYNQENWDQLLQQLSNNHQAIPVINRAQIIDDAFNLARAQQVSVTLALNTTRFLSGETAYMPWQAALNNLQYFQLMFDRSEVFGAMTKYIQKQVTPLFEYYRTATNNWTAIPSALMDQYNEINAISTACSYGIAECQQLATALYQQWRQNVSNNPIAPNLRSAIYCSAVATGGEEVWDFIWERFLEAPVVSEADKLRTALTCSTETWILQRYLQYTIDPTKIRKQDATSTINSIASNVVGQPLAWDFIRSNWRTLFGQYGGGSFSFSRLISAVTQRFNTEFELKQLEQFKADNQDIGFGSGTRALEQALERTRTNINWVKENKEVVHAWFRAETASS

SEQ ID NO: 7 - protein, 150 aa, Gallus gallus
MAFHSTLLVFLAGLVFLSEAAPLVSHGSVDSKCPLMVKVLDAVRGSPAANVAVKVFKKAADGTWQDFATGKTTEFGEIHELTTEEQFVEGVYRVEFDTSSYWKGLGLSPFHEYADVVFTANDSGHRHYTIAALLSPFSYSTTAVVSDPQE

SEQ ID NO: 8 - protein, 472 aa, Gallus gallus
MRTARQFVQVALALCCFADIAFGIEVNCSLYASGIGKDGTSWVACPRNLKPVCGTDGSTYSNECGICLYNREHGANVEKEYDGECRPKHVMIDCSPYLQVVRDGNTMVACPRILKPVCGSDSFTYDNECGICAYNAEHHTNISKLHDGECKLEIGSVDCSKYPSTVSKDGRTLVACPRILSPVCGTDGFTYDNECGICAHNAEQRTHVSKKHDGKCRQEIPEIDCDQYPTRKTTGGKLLVRCPRILLPVCGTDGFTYDNECGICAHNAQHGTEVKKSHDGRCKERSTPLDCTQYLSNTQNGEAITACPFILQEVCGTDGVTYSNDCSLCAHNIELGTSVAKKHDGRCREEVPELDCSKYKTSTLKDGRQVVACTMIYDPVCATNGVTYASECTLCAHNLEQRTNLGKRKNGRCEEDITKEHCREFQKVSPICTMEYVPHCGSDGVTYSNRCFFCNAYVQSNRTLNLVSMAAC

SEQ ID NO: 9 - protein, 264 aa, Gallus gallus
MRGVLVTLAVLFLTGTQARSFWQHDEPQTPLDRIRDMVDVYLETVKASGKDAIAQFESSAVGKQLDLKLADNLDTLSAAAAKLREDMAPYYKEVREMWLKDTEALRAELTKDLEEVKEKIRPFLDQFSAKWTEELEQYRQRLTPVAQELKELTKQKVELMQAKLTPVAEEARDRLRGHVEELRKNLAPYSDELRQKLSQKLEEIREKGIPQASEYQAKVMEQLSNLREKMTPLVQEFRERLTPYAENLKNRLISFLDELQKSVA

SEQ ID NO: 10 - protein, 12 aa, Gallus gallus
APFSGELSGPVK

SEQ ID NO: 11 - protein, 12 aa, Gallus gallus
APFSGQLSGPIR

SEQ ID NO: 12 - protein, 10 aa, Gallus gallus
FSGELSGPVK

SEQ ID NO: 13 - protein, 6 aa, Gallus gallus
HGQIQK

SEQ ID NO: 14 - protein, 9 aa, Gallus gallus
SDPTSNLER

SEQ ID NO: 15 - protein, 9 aa, Gallus gallus
SGELSGPVK

SEQ ID NO: 16 - protein, 9 aa, Gallus gallus
SGQLSGPIR

SEQ ID NO: 17 - protein, 9 aa, Gallus gallus
VFPGIISHI

SEQ ID NO: 18 - protein, 8 aa, Gallus gallus
VFPGIVSH

SEQ ID NO: 19 - protein, 9 aa, Gallus gallus
VFPGIVSHI

SEQ ID NO: 20 - protein, 7 aa, Gallus gallus
ATITGYK

SEQ ID NO: 21 - protein, 10 aa, Gallus gallus
DDQESIPISK

SEQ ID NO: 22 - protein, 15 aa, Gallus gallus
KAMKGMGTDEETILK

SEQ ID NO: 23 - protein, 7 aa, Gallus gallus
LLLAVVK

SEQ ID NO: 24 - protein, 8 aa, Gallus gallus
VDEALVEK

SEQ ID NO: 25 - protein, 7 aa, Gallus gallus
IGNASTK

SEQ ID NO: 26 - protein, 5 aa, Gallus gallus
TPDSK

SEQ ID NO: 27 - protein, 9 aa, Gallus gallus
TVTLGAGAK

SEQ ID NO: 28 - protein, 7 aa, Gallus gallus
VVLASLK

SEQ ID NO: 29 - protein, 10 aa, Gallus gallus
VGNAKPEIQK

SEQ ID NO: 30 - protein, 11 aa, Gallus gallus
VVDALNSIQTK

SEQ ID NO: 31 - protein, 13 aa, Gallus gallus
ADNQDIGFGSGTR

SEQ ID NO: 32 - protein, 13 aa, Gallus gallus
AIAEGQGEYALEK

SEQ ID NO: 33 - protein, 9 aa, Gallus gallus
APVVSEADK

SEQ ID NO: 34 - protein, 12 aa, Gallus gallus
AQIIDDAFNLAR

SEQ ID NO: 35 - protein, 11 aa, Gallus gallus
AVFTVTMIHPS

SEQ ID NO: 36 - protein, 6 aa, Gallus gallus
AWDFIR

SEQ ID NO: 37 - protein, 6 aa, Gallus gallus
DFIWER

SEQ ID NO: 38 - protein, 9 aa, Gallus gallus
DFLTEDVFK

SEQ ID NO: 39 - protein, 9 aa, Gallus gallus
DHLQEAVNK

SEQ ID NO: 40 - protein, 12 aa, Gallus gallus
DLWDHLQEAVNK

SEQ ID NO: 41 - protein, 10 aa, Gallus gallus
DNAYSSIGNK

SEQ ID NO: 42 - protein, 10 aa, Gallus gallus
EAPVVSEADK

SEQ ID NO: 43 - protein, 10 aa, Gallus gallus
EGQGEYALEK

SEQ ID NO: 44 - protein, 16 aa, Gallus gallus
ENSLLYDNAYSSIGNK

SEQ ID NO: 45 - protein, 6 aa, Gallus gallus
EQALER

SEQ ID NO: 46 - protein, 12 aa, Gallus gallus
FLEAPVVSEADK

SEQ ID NO: 47 - protein, 14 aa, Gallus gallus
FLEAPVVSEADKLR

SEQ ID NO: 48 - protein, 8 aa, Gallus gallus
FNTEFELK

SEQ ID NO: 49 - protein, 12 aa, Gallus gallus
GADSAEPTWDIK

SEQ ID NO: 50 - protein, 10 aa, Gallus gallus
HYNTAYPLPK

SEQ ID NO: 51 - protein, 12 aa, Gallus gallus
IAEGQGEYALEK

SEQ ID NO: 52 - protein, 7 aa, Gallus gallus
ILSFFER

SEQ ID NO: 53 - protein, 10 aa, Gallus gallus
IWGRPAAIAE

SEQ ID NO: 54 - protein, 15 aa, Gallus gallus
IWGRPAAIAEGQGEY

SEQ ID NO: 55 - protein, 19 aa, Gallus gallus
IWGRPAAIAEGQGEYALEK

SEQ ID NO: 56 - protein, 9 aa, Gallus gallus
KQDATSTIN

SEQ ID NO: 57 - protein, 20 aa, Gallus gallus
KQDATSTINSIASNVVGQPL

SEQ ID NO: 58 - protein, 21 aa, Gallus gallus
KQDATSTINSIASNVVGQPLA

SEQ ID NO: 59 - protein, 12 aa, Gallus gallus
LAGPLQQGQHYR

SEQ ID NO: 60 - protein, 11 aa, Gallus gallus
LEAPVVSEADK

SEQ ID NO: 61 - protein, 17 aa, Gallus gallus
LPTALKPESYEVTLQPF

SEQ ID NO: 62 - protein, 12 aa, Gallus gallus
MLSDFLTEDVFK

SEQ ID NO: 63 - protein, 15 aa, Gallus gallus
NSVPLPDSIGAIMDR

SEQ ID NO: 64 - protein, 15 aa, Gallus gallus
PAAIAEGQGEYALEK

SEQ ID NO: 65 - protein, 8 aa, Gallus gallus
QAIPVINR

SEQ ID NO: 66 - protein, 19 aa, Gallus gallus
QDATSTINSIASNVVGQPL

SEQ ID NO: 67 - protein, 13 aa, Gallus gallus
QNVSNNPIAPNLR

SEQ ID NO: 68 - protein, 10 aa, Gallus gallus
SDFLTEDVFK

SEQ ID NO: 69 - protein, 18 aa, Gallus gallus
SDQVGLPDFNAGAMENWG

SEQ ID NO: 70 - protein, 11 aa, Gallus gallus
SEVFDSIAYSK

SEQ ID NO: 71 - protein, 14 aa, Gallus gallus
SLLYDNAYSSIGNK

SEQ ID NO: 72 - protein, 12 aa, Gallus gallus
SNNHQAIPVINR

SEQ ID NO: 73 - protein, 14 aa, Gallus gallus
SVPLPDSIGAIMDR

SEQ ID NO: 74 - protein, 13 aa, Gallus gallus
TDLWDHLQEAVNK

SEQ ID NO: 75 - protein, 13 aa, Gallus gallus
TGELADDLAGFYR

SEQ ID NO: 76 - protein, 10 aa, Gallus gallus
TGPILSFFER

SEQ ID NO: 77 - protein, 6 aa, Gallus gallus
TIDPTK

SEQ ID NO: 78 - protein, 15 aa, Gallus gallus
TLFGQYGGGSFSFSR

SEQ ID NO: 79 - protein, 7 aa, Gallus gallus
TNINWVK

SEQ ID NO: 80 - protein, 12 aa, Gallus gallus
VNYNQENWDQLL

SEQ ID NO: 81 - protein, 13 aa, Gallus gallus
VNYNQENWDQLLQ

SEQ ID NO: 82 - protein, 14 aa, Gallus gallus
VNYNQENWDQLLQQ

SEQ ID NO: 83 - protein, 13 aa, Gallus gallus
VVATTQMQAPDAR

SEQ ID NO: 84 - protein, 7 aa, Gallus gallus
WRLPTAL

SEQ ID NO: 85 - protein, 11 aa, Gallus gallus
WRLPTALKPES

SEQ ID NO: 86 - protein, 19 aa, Gallus gallus
WRLPTALKPESYEVTLQPF

SEQ ID NO: 87 - protein, 11 aa, Gallus gallus
YDNAYSSIGNK

SEQ ID NO: 88 - protein, 10 aa, Gallus gallus
YLQYTIDPTK

SEQ ID NO: 89 - protein, 5 aa, Gallus gallus
YPLPK

SEQ ID NO: 90 - protein, 13 aa, Gallus gallus
AADGTWQDFATGK

SEQ ID NO: 91 - protein, 6 aa, Gallus gallus
CPLMVK

SEQ ID NO: 92 - protein, 11 aa, Gallus gallus
DGTWQDFATGK

SEQ ID NO: 93 - protein, 12 aa, Gallus gallus
DVVFTANDSGHR

SEQ ID NO: 94 - protein, 8 aa, Gallus gallus
GLGLSPFH

SEQ ID NO: 95 - protein, 10 aa, Gallus gallus
GLGLSPFHEY

SEQ ID NO: 96 - protein, 11 aa, Gallus gallus
GLGLSPFHEYA

SEQ ID NO: 97 - protein, 15 aa, Gallus gallus
GLGLSPFHEYADVVF

SEQ ID NO: 98 - protein, 23 aa, Gallus gallus
GLGLSPFHEYADVVFTANDSGHR

SEQ ID NO: 99 - protein, 10 aa, Gallus gallus
GSPAANVAVK

SEQ ID NO: 100 - protein, 11 aa, Gallus gallus
GSPAANVAVKV

SEQ ID NO: 101 - protein, 10 aa, Gallus gallus
GTWQDFATGK

SEQ ID NO: 102 - protein, 8 aa, Gallus gallus
HYTIAALL

SEQ ID NO: 103 - protein, 11 aa, Gallus gallus
HYTIAALLSPF

SEQ ID NO: 104 - protein, 12 aa, Gallus gallus
HYTIAALLSPFS

SEQ ID NO: 105 - protein, 12 aa, Gallus gallus
TTEEQFVEGVYR

SEQ ID NO: 106 - protein, 10 aa, Gallus gallus
TTEFGEIHEL

SEQ ID NO: 107 - protein, 15 aa, Gallus gallus
TTEFGEIHELTTEEQ

SEQ ID NO: 108 - protein, 20 aa, Gallus gallus
TTEFGEIHELTTEEQFVEGV

SEQ ID NO: 109 - protein, 22 aa, Gallus gallus
TTEFGEIHELTTEEQFVEGVYR

SEQ ID NO: 110 - protein, 32 aa, Gallus gallus
TTEFGEIHELTTEEQFVEGVYRVEFDTSSYWK

SEQ ID NO: 111 - protein, 10 aa, Gallus gallus
VEFDTSSYWK

SEQ ID NO: 112 - protein, 6 aa, Gallus gallus
VLDAVR

SEQ ID NO: 113 - protein, 8 aa, Gallus gallus
EHGANVEK

SEQ ID NO: 114 - protein, 10 aa, Gallus gallus
TLNLVSMAAC

SEQ ID NO: 115 - protein, 7 aa, Gallus gallus
TLVACPR

SEQ ID NO: 116 - protein, 8 aa, Gallus gallus
DLEEVKEK

SEQ ID NO: 117 - protein, 5 aa, Gallus gallus
EMWLK

SEQ ID NO: 118 - protein, 7 aa, Gallus gallus
IRDMVDV

SEQ ID NO: 119 - protein, 8 aa, Gallus gallus
IRPFLDQF

SEQ ID NO: 120 - protein, 11 aa, Gallus gallus
IRPFLDQFSAK

SEQ ID NO: 121 - protein, 14 aa, Gallus gallus
LADNLDTLSAAAAK

SEQ ID NO: 122 - protein, 10 aa, Gallus gallus
LISFLDELQK

SEQ ID NO: 123 - protein, 8 aa, Gallus gallus
LSQKLEEI

SEQ ID NO: 124 - protein, 9 aa, Gallus gallus
LTPVAEEAR

SEQ ID NO: 125 - protein, 9 aa, Gallus gallus
LTPVAQELK

SEQ ID NO: 126 - protein, 9 aa, Gallus gallus
LTPYAENLK

SEQ ID NO: 127 - protein, 9 aa, Gallus gallus
MTPLVQEFR

SEQ ID NO: 128 - protein, 6 aa, Gallus gallus
QKLSQK

SEQ ID NO: 129 - protein, 5 aa, Gallus gallus
QLDLK

SEQ ID NO: 130 - protein, 5 aa, Gallus gallus
YKEVR

SEQ ID NO: 131 - protein, 147 aa, Gallus gallus
MVHWTAEEKQLITGLWGKVNVAECGAEALARLLIVYPWTQRFFASFGNLSSPTAILGNPMVRAHGKKVLTSFGDAVKNLDNIKNTFSQLSELHCDKLHVDPENFRLLGDILIIVLAAHFSKDFTPECQAAWQKLVRVVAHALARKYH

SEQ ID NO: 132 - protein, 154 aa, Gallus gallus
MATLKAVCVMKGDAPVEGVIHFQQQGSGPVKVTGKITGLSDGDHGFHVHEFGDNTNGCTSAGAHFNPEGKQHGGPKDADRHVGDLGNVTAKGGVAEVEIEDSVISLTGPHCIIGRTMVVHAKSDDLGRGGDNESKLTGNAGPRLACGVIGIAKC

SEQ ID NO: 133 - protein, 904 aa, Gallus gallus
MVDYHSAGQPYPYGGNGPGPNGDYMAQEDDWDRDLLLDPAWEKQQRKTFTAWCNSHLRKAGTQIENIDEDFRDGLKLMLLLEVISGERLPKPERGKMRVHKINNVNKALDFIASKGVNVVSIGAEEIVDGNAKMTLGMIWTIILRFAIQDISVEETSAKEGLLLWCQRKTAPYKNVNVQNFHISWKDGLAFNALIHRHRPELIEYDKLRKDDPVTNLNNAFEVAEKYLDIPKMLDAEDIVNTARPDEKAIMTYVSSFYHAFSGAQKAETAANRICKVLAVNQENEHLMEDYEKLASDLLEWIRRTIPWLEDRSPQKTIQEMQQKLEDFRDYRRVHKPPKVQEKCQLEINFNTLQTKLRLSNRPAFMPSEGRMVSDINTGWQHLEQAEKGYEEWLLNEIRRLEPLDHLAEKFRQKASIHEAWTEGKEAMLKQKDYETATLSDIKALIRKHEAFESDLAAHQDRVEQIAAIAQELNELDYYDSPSVNARCQKICDQWDVLGSLTHSRREALEKTEKQLETIDELHLEYAKRAAPFNNWMESAMEDLQDMFIVHTIEEIEGLIAAHDQFKATLPDADREREAILGIQREAQRIADLHSIKLSGNNPYTSVTPQVINSKWERVQQLVPTRDRALQDEQSRQQCNERLRRQFAGQANIVGPWMQTKMEEIGRISIEMHGTLEDQLQHLKHYEQSIVDYKPNLELLEHEHQLVEEALIFDNKHTNYTMEHIRVGWEQLLTTIARTINEVENQILTRDAKGISQEQMQEFRASFNHFDKDHCGALGPEEFKACLISLGYDVENDRQGDAEFNRIMSLVDPNGSGSVTFQAFIDFMSRETTDTDTADQVIASFKVLAGDKNYITAEELRRELPPEQAEYCIARMAPYRGPDAAPGALDYKSFSTALYGESDL

SEQ ID NO: 134 - protein, 1193 aa, Gallus gallus
AKELYGNIWSNFSDPQLKKIIGSIQTLGPSNLPLDKRQQYNTILSDMDKIYSTAKVCLDNGTCWDLEPDISDIMATSRSYKKLLYAWEGWHNAAGNPLRAKYQEFVTLSNEAYQMDGFEDTGSYWRSWYDSTTFEDDLEHLYNQLEPLYLNLHAFVRRKLYDRYGPKYINLKGPIPAHLLGNMWAQQWNNIYDLMVPYPDKPNLDVTNTMVNQGWNATHMFRVSEEFFTSLGLLEMPPEFWEKSMLEKPADGREVVCHASAWDFYNRKDFRIKQCTTVTMEQLFTVHHEMGHVQYYLQYKDQPVSFRGGANPGFHEAIGDVLSLSVSTPSHLQKIGLLSSAVEDEESNINYLLKMALEKIAFLPFGYLIDQWRWNVFSGRTPPSRYNYDWWYLRTKYQGICAPVSRNESNFDPGAKYHIPGNTPYIRYFVSFILQFQFHKALCQAANHTGPLHTCDIYMSKEAGAKLREVLKAGSSKSWQEILFNLTGTDKMDAGALLEYFSPVTTWLQEQNNKTNEVLGWPEFDWRSPIPEGYPEGIDKIVDEAQAKEFLSEYNSTAEVVWNAYTEASWEYNTNITDHNKEVMLEKNLAMSKHTIEYGMRARQFDPSDFQDETVTRILNKLSVLERAALPEDELKEYNTLLSDMETTYSVAKVCRENNTFHPLDPDLTDILATSRDYNELLFAWKGWWDASGAKIKDKYKRYVELSNKAAVLNGYTDNGAYWRSLYETPTFEEDLERLYLQLQPLYLNLHAYVRRALYNKYGAEHISLKGPIPAHLLGNMWAQSWSNIFDLVMPFPDATKVDATPAMKQQGWTPKMMFEESDRFFTSLGLIPMPQEFWDKSMIEKPADGREVVCHASAWDFYNRKDFRIKQCTVVNMDDLITVHHEMGHVQYFLQYMDQPISFRDGANPGFHEAIGDVMALSVSTPKHLHSINLLDQVTENEESDINYLMSIALDKIAFLPFGYLMDQWRWKVFDGRIKEDEYNQQWWNLRLKYQGLCPPVPRSEDDFDPGAKFHIPANVPYIRYFVSFVIQFQFHQALCKAAGHTGPLHTCDIYQSKEAGKLLGDAMKLGFSKPWPEAMQLITGQPNMSAEALMSYFEPLMTWLVKKNTENGEVLGWPEYSWTPYAVTEFHAATDTADFLGMSVGTKQATAGAWVLLALALVFLITSIFLGVKLFSSRRKAFKSSSEMELK

SEQ ID NO: 135 - protein, 609 aa, Gallus gallus
MRMPYEIKKVFASLPQVERGVSKIIGGDPKGNNFLYTNGKCVVIRNIDNPAIADIYTEHAHQVVVAKYAPSGFYIASGDVSGKLRIWDTTQKEHLLKYEYQPFAGKIKDLAWTEDSKRIAVVGEGREKFGAVFLWDSGSSVGEITGHNKVINSVDIKQTRPYRLATGSDDNCAAFFEGPPFKFKFTLSDHTRFVNCVRFSPDGNRFATASADGQIFIYDGKTGEKVCALGGGKAHDGGIYAISWSPDSSQLLSASGDKTAKIWDVGANSVVSTFNMGSNVLDQQLGCLWQKDHLLSLSLSGYINYLDKNNPDKPLRVIKGHSKSIQCLTVHKNGGKSYIYSGSNDGHINYWDSDTGENDGFSGKGHTNQVSRMAVDEMDQLVTCSMDDTVRYTNLSKRDYSGQDAVKMDVQPKCLAVGPGGYTVVLCIGQIVLMKDKKKCFAIDDLGYEPEAVAVHPGGGSVAVGGTDGNVRLYSIQGTSLKSDDKTLEAKGPVTDLAYSHDGAFLAVCDANKVVTVFSVPDGYVEHNVFYGHHAKVVCIAWSPDNEHFASGGMDMMVYVWTVSDPETRIKIPDAHRLHHVSGLAWLDEHTLVTTSHDASVKEWSISYN

SEQ ID NO: 136 - protein, 423 aa, Gallus gallus
MALLQSRLLLSAPRRAAATARASSWWSHVEMGPPDPILGVTEAFKRDTNSKKMNLGVGAYRDDNGKSYVLNCVRKAEAMIAAKKMDKEYLPIAGLADFTRASAELALGENSEAFKSGRYVTVQGISGTGSLRVGANFLQRFFKFSRDVYLPKPSWGNHTPIFRDAGLQLQAYRYYDPKTCSLDFTGAMEDISKIPEKSIILLHACAHNPTGVDPRQEQWKELASVVKKRNLLAYFDMAYQGFASGDINRDAWALRHFIEQGIDVVLSQSYAKNMGLYGERAGAFTVICRDAEEAKRVESQLKILIRPMYSNPPMNGARIASLILNTPELRKEWLVEVKGMADRIISMRTQLVSNLKKEGSSHNWQHITDQIGMFCFTGLKPEQVERLTKEFSIYMTKDGRISVAGVASSNVGYLAHAIHQVTK

SEQ ID NO: 137 - protein, 129 aa, Gallus gallus
MSGRGKQGGKARAKAKSRSSRAGLQFPVGRVHRLLRKGNYAERVGAGAPVYLAAVLEYLTAEILELAGNAARDNKKTRIIPRHLQLAIRNDEELNKLLGKVTIAQGGVLPNIQAVLLPKKTDSHKAKAK

SEQ ID NO: 138 - protein, 103 aa, Gallus gallus
QPKVAPTITLFPPSKEELNEATKATLVCLINDFYPSPVTVDWVIDGSTRSGETTAPQRQSNSQYMASSYLSLSASDWSSHETYTCRVTHNGTSITKTLKRSEC

SEQ ID NO: 139 - protein, 113 aa, Gallus gallus
MAWAPLLLAVLAHTSGSLVQAALTQPSSVSANPGETVKITCSGDRSYYGWYQQKAPGSAPVTLIYDNTNRPSNIPSRFSGSKSGSTATLTITGVQADDEAVYYCGSADSSSTA

SEQ ID NO: 140 - protein, 398 aa, Gallus gallus
MAPRGLLVLLLLALVGPCAALIRIPLTKFTSTRRMLTEVGSEIPDMNAITQFLKFKLGFADLAEPTPEILKNYMDAQYYGEIGIGTPPQKFTVVFDTGSSNLWVPSVHCHLLDIACLLHHKYDASKSSTYVENGTEFAIHYGTGSLSGFLSQDTVTLGNLKIKNQIFGEAVKQPGITFIAAKFDGILGMAFPRISVDKVTPFFDNVMQQKLIEKNIFSFYLNRDPTAQPGGELLLGGTDPKYYSGDFSWVNVTRKAYWQVHMDSVDVANGLTLCKGGCEAIVDTGTSLITGPTKEVKELQTAIGAKPLIKGQYVISCDKISSLPVVTLMLGGKPYQLTGEQYVFKVSAQGETICLSGFSGLDVPPPGGPLWILGDVFIGPYYTVFDRDNDSVGFAKCV

SEQ ID NO: 141 - protein, 196 aa, Gallus gallus
MAYTWRALLLLALAFLGSSMAERDCRVSSFKVKENFDKNRYSGTWYAMAKKDPEGLFLQDNVVAQFTVDENGQMSATAKGRVRLFNNWDVCADMIGSFTDTEDPAKFKMKYWGVASFLQKGNDDHWVVDTDYDTYALHYSCRELNEDGTCADSYSFVFSRDPKGLPPEAQKIVRQRQIDLCLDRKYRVIVHNGFCS

SEQ ID NO: 142 - protein, 10 aa, Gallus gallus
KVLTSFGDAV

SEQ ID NO: 143 - protein, 8 aa, Gallus gallus
LHVDPENF

SEQ ID NO: 144 - protein, 10 aa, Gallus gallus
LLIVYPWTQR

SEQ ID NO: 145 - protein, 6 aa, Gallus gallus
NLDNIK

SEQ ID NO: 146 - protein, 10 aa, Gallus gallus
VLTSFGDAVK

SEQ ID NO: 147 - protein, 6 aa, Gallus gallus
AVCVMK

SEQ ID NO: 148 - protein, 10 aa, Gallus gallus
FQQQGSGPVK

SEQ ID NO: 149 - protein, 20 aa, Gallus gallus
GDAPVEGVIHFQQQGSGPVK

SEQ ID NO: 150 - protein, 8 aa, Gallus gallus
GGVAEVEI

SEQ ID NO: 151 - protein, 19 aa, Gallus gallus
GGVAEVEIEDSVISLTGPH

SEQ ID NO: 152 - protein, 7 aa, Gallus gallus
GVIGIAK

SEQ ID NO: 153 - protein, 10 aa, Gallus gallus
HVGDLGNVTA

SEQ ID NO: 154 - protein, 11 aa, Gallus gallus
HVGDLGNVTAK

SEQ ID NO: 155 - protein, 14 aa, Gallus gallus
ITGLSDGDHGFHVH

SEQ ID NO: 156 - protein, 10 aa, Gallus gallus
LACGVIGIAK

SEQ ID NO: 157 - protein, 8 aa, Gallus gallus
LTGNAGPR

SEQ ID NO: 158 - protein, 6 aa, Gallus gallus
SDDLGR

SEQ ID NO: 159 - protein, 13 aa, Gallus gallus
SDDLGRGGDNESK

SEQ ID NO: 160 - protein, 6 aa, Gallus gallus
TMVVHA

SEQ ID NO: 161 - protein, 14 aa, Gallus gallus
DAEDIVNTARPDEK

SEQ ID NO: 162 - protein, 8 aa, Gallus gallus
TIPWLEDR

SEQ ID NO: 163 - protein, 26 aa, Gallus gallus
AALPEDELKEYNTLLSDMETTYSVAK

SEQ ID NO: 164 - protein, 5 aa, Gallus gallus
ALYNK

SEQ ID NO: 165 - protein, 14 aa, Gallus gallus
DGANPGFHEAIGDV

SEQ ID NO: 166 - protein, 16 aa, Gallus gallus
DGANPGFHEAIGDVMA

SEQ ID NO: 167 - protein, 17 aa, Gallus gallus
DGANPGFHEAIGDVMAL

SEQ ID NO: 168 - protein, 10 aa, Gallus gallus
DYNELLFAWK

SEQ ID NO: 169 - protein, 11 aa, Gallus gallus
ETPTFEEDLER

SEQ ID NO: 170 - protein, 6 aa, Gallus gallus
EVMLEK

SEQ ID NO: 171 - protein, 6 aa, Gallus gallus
FEESDR

SEQ ID NO: 172 - protein, 17 aa, Gallus gallus
FFTSLGLIPMPQEFWDK

SEQ ID NO: 173 - protein, 16 aa, Gallus gallus
GGANPGFHEAIGDVLS

SEQ ID NO: 174 - protein, 12 aa, Gallus gallus
GLIPMPQEFWDK

SEQ ID NO: 175 - protein, 12 aa, Gallus gallus
GLLEMPPEFWEK

SEQ ID NO: 176 - protein, 7 aa, Gallus gallus
GPIPAHL

SEQ ID NO: 177 - protein, 12 aa, Gallus gallus
GPIPAHLLGNMW

SEQ ID NO: 178 - protein, 15 aa, Gallus gallus
GPIPAHLLGNMWAQQ

SEQ ID NO: 179 - protein, 15 aa, Gallus gallus
GPIPAHLLGNMWAQS

SEQ ID NO: 180 - protein, 8 aa, Gallus gallus
GYLIDQWR

SEQ ID NO: 181 - protein, 17 aa, Gallus gallus
IIGSIQTLGPSNLPLDK

SEQ ID NO: 182 - protein, 18 aa, Gallus gallus
IIGSIQTLGPSNLPLDKR

SEQ ID NO: 183 - protein, 13 aa, Gallus gallus
IKEDEYNQQWWNL

SEQ ID NO: 184 - protein, 18 aa, Gallus gallus
KIIGSIQTLGPSNLPLDK

SEQ ID NO: 185 - protein, 18 aa, Gallus gallus
KIIGSIQTLGPSNLPLDK

SEQ ID NO: 186 - protein, 7 aa, Gallus gallus
LLGDAMK

SEQ ID NO: 187 - protein, 17 aa, Gallus gallus
LLYAWEGWHNAAGNPLR

SEQ ID NO: 188 - protein, 6 aa, Gallus gallus
LSVLER

SEQ ID NO: 189 - protein, 7 aa, Gallus gallus
MSIALDK

SEQ ID NO: 190 - protein, 9 aa, Gallus gallus
NTILSDMDK

SEQ ID NO: 191 - protein, 14 aa, Gallus gallus
QCTVVNMDDLITVH

SEQ ID NO: 192 - protein, 14 aa, Gallus gallus
QFDPSDFQDETVTR

SEQ ID NO: 193 - protein, 7 aa, Gallus gallus
QQGWTPK

SEQ ID NO: 194 - protein, 12 aa, Gallus gallus
QQYNTILSDMDK

SEQ ID NO: 195 - protein, 8 aa, Gallus gallus
RYVELSNK

SEQ ID NO: 196 - protein, 14 aa, Gallus gallus
SLGLIPMPQEFWDK

SEQ ID NO: 197 - protein, 12 aa, Gallus gallus
SLSVSTPSHLQK

SEQ ID NO: 198 - protein, 14 aa, Gallus gallus
SLYETPTFEEDLER

SEQ ID NO: 199 - protein, 10 aa, Gallus gallus
SMIEKPADGR

SEQ ID NO: 200 - protein, 15 aa, Gallus gallus
SNIFDLVMPFPDATK

SEQ ID NO: 201 - protein, 6 aa, Gallus gallus
SVSTPK

SEQ ID NO: 202 - protein, 10 aa, Gallus gallus
SVSTPSHLQK

SEQ ID NO: 203 - protein, 11 aa, Gallus gallus
TLGPSNLPLDK

SEQ ID NO: 204 - protein, 26 aa, Gallus gallus
TNEVLGWPEFDWRSPIPEGYPEGIDK

SEQ ID NO: 205 - protein, 15 aa, Gallus gallus
TSLGLIPMPQEFWDK

SEQ ID NO: 206 - protein, 15 aa, Gallus gallus
TSLGLLEMPPEFWEK

SEQ ID NO: 207 - protein, 8 aa, Gallus gallus
VDATPAMK

SEQ ID NO: 208 - protein, 6 aa, Gallus gallus
VELSNK

SEQ ID NO: 209 - protein, 9 aa, Gallus gallus
YGAEHISLK

SEQ ID NO: 210 - protein, 9 aa, Gallus gallus
YHIPGNTPY

SEQ ID NO: 211 - protein, 5 aa, Gallus gallus
YINLK

SEQ ID NO: 212 - protein, 9 aa, Gallus gallus
YNELLFAWK

SEQ ID NO: 213 - protein, 10 aa, Gallus gallus
YQGLCPPVPR

SEQ ID NO: 214 - protein, 7 aa, Gallus gallus
YVELSNK

SEQ ID NO: 215 - protein, 7 aa, Gallus gallus
IIGGDPK

SEQ ID NO: 216 - protein, 15 aa, Gallus gallus
KVFASLPQVERGVSK

SEQ ID NO: 217 - protein, 8 aa, Gallus gallus
VINSVDIK

SEQ ID NO: 218 - protein, 14 aa, Gallus gallus
GPPDPILGVTEAFK

SEQ ID NO: 219 - protein, 7 aa, Gallus gallus
LLLSAPR

SEQ ID NO: 220 - protein, 8 aa, Gallus gallus
MDKEYLPI

SEQ ID NO: 221 - protein, 7 aa, Gallus gallus
MGLYGER

SEQ ID NO: 222 - protein, 8 aa, Gallus gallus
NPTGVDPR

SEQ ID NO: 223 - protein, 8 aa, Gallus gallus
TQLVSNLK

SEQ ID NO: 224 - protein, 7 aa, Gallus gallus
NDEELNK

SEQ ID NO: 225 - protein, 19 aa, Gallus gallus
VTIAQGGVLPNIQAVLLPK

SEQ ID NO: 226 - protein, 18 aa, Gallus gallus
DFYPSPVTVDWVIDGSTR

SEQ ID NO: 227 - protein, 8 aa, Gallus gallus
ITLFPPSK

SEQ ID NO: 228 - protein, 19 aa, Gallus gallus
NDFYPSPVTVDWVIDGSTR

SEQ ID NO: 229 - protein, 9 aa, Gallus gallus
SGETTAPQR

SEQ ID NO: 230 - protein, 9 aa, Gallus gallus
THNGTSITK

SEQ ID NO: 231 - protein, 11 aa, Gallus gallus
TVDWVIDGSTR

SEQ ID NO: 232 - protein, 12 aa, Gallus gallus
VAPTITLFPPSK

SEQ ID NO: 233 - protein, 16 aa, Gallus gallus
VAPTITLFPPSKEELN

SEQ ID NO: 234 - protein, 19 aa, Gallus gallus
VAPTITLFPPSKEELNEAT

SEQ ID NO: 235 - protein, 20 aa, Gallus gallus
VAPTITLFPPSKEELNEATK

SEQ ID NO: 236 - protein, 10 aa, Gallus gallus
VTHNGTSITK

SEQ ID NO: 237 - protein, 17 aa, Gallus gallus
ALTQPSSVSANPGETVK

SEQ ID NO: 238 - protein, 23 aa, Gallus gallus
APGSAPVTLIYDNTNRPSNIPSR

SEQ ID NO: 239 - protein, 21 aa, Gallus gallus
GSAPVTLIYDNTNRPSNIPSR

SEQ ID NO: 240 - protein, 7 aa, Gallus gallus
ITCSGDR

SEQ ID NO: 241 - protein, 7 aa, Gallus gallus
NPGETVK

SEQ ID NO: 242 - protein, 7 aa, Gallus gallus
PSNIPSR

SEQ ID NO: 243 - protein, 8 aa, Gallus gallus
RPSNIPSR

SEQ ID NO: 244 - protein, 9 aa, Gallus gallus
SANPGETVK

SEQ ID NO: 245 - protein, 11 aa, Gallus gallus
SVSANPGETVK

SEQ ID NO: 246 - protein, 7 aa, Gallus gallus
YGWYQQK

SEQ ID NO: 247 - protein, 18 aa, Gallus gallus
DPTAQPGGELLLGGTDPK

SEQ ID NO: 248 - protein, 11 aa, Gallus gallus
ELQTAIGAKPL

SEQ ID NO: 249 - protein, 12 aa, Gallus gallus
ELQTAIGAKPLI

SEQ ID NO: 250 - protein, 11 aa, Gallus gallus
FDGILGMAFPR

SEQ ID NO: 251 - protein, 5 aa, Gallus gallus
IPLTK

SEQ ID NO: 252 - protein, 14 aa, Gallus gallus
QPGGELLLGGTDPK

SEQ ID NO: 253 - protein, 12 aa, Gallus gallus
VTPFFDNVMQQK

SEQ ID NO: 254 - protein, 8 aa, Gallus gallus
QIDLCLDR

SEQ ID NO: 255 - protein, 13 aa, Gallus gallus
TVDENGQMSATAK